European Patent Application EP 4 123 021 A1, published January 25, 2023. Title: ANTI-TUMOR ADENOVIRUS. Applicant: Curigin Co., Ltd. The sequence listing filed with the application follows.

SEQUENCE LISTING (82 sequences)

SEQ ID NO: 1 - RNA, 21 nt, Artificial Sequence
  si-MS1
gacuguggcauccaccugcau

SEQ ID NO: 2 - RNA, 21 nt, Artificial Sequence
  si-MS1 antisense
augcagguaggcgccucaguc

SEQ ID NO: 3 - RNA, 20 nt, Artificial Sequence
  si-MS2 sense
gacuguggcauccaccugca

SEQ ID NO: 4 - RNA, 20 nt, Artificial Sequence
  si-MS2 antisense
ugcagguaggcgccucaguc

SEQ ID NO: 5 - RNA, 19 nt, Artificial Sequence
  si-MS3 sense
gacuguggcauccaccugc

SEQ ID NO: 6 - RNA, 19 nt, Artificial Sequence
  si-MS3 antisense
gcagguaggcgccucaguc

SEQ ID NO: 7 - RNA, 18 nt, Artificial Sequence
  si-MS4 sense
gacuguggcauccaccug

SEQ ID NO: 8 - RNA, 18 nt, Artificial Sequence
  si-MS4 antisense
cagguaggcgccucaguc

SEQ ID NO: 9 - RNA, 17 nt, Artificial Sequence
  si-MS5 sense
ucagccacagcagcuug

SEQ ID NO: 10 - RNA, 17 nt, Artificial Sequence
  si-MS5 antisense
caagcugcuguagcuga

SEQ ID NO: 11 - RNA, 20 nt, Artificial Sequence
  si-MS6 sense
gcagcgcaugcggcccagca

SEQ ID NO: 12 - RNA, 20 nt, Artificial Sequence
  si-MS6 antisense
ugcugggccgcaguggcugc

SEQ ID NO: 13 - RNA, 19 nt, Artificial Sequence
  si-MS7 sense
gcagcgcaugcggcccagc

SEQ ID NO: 14 - RNA, 19 nt, Artificial Sequence
  si-MS7 antisense
gcugggccgcaguggcugc

SEQ ID NO: 15 - RNA, 18 nt, Artificial Sequence
  si-MS8 sense
gcagcgcaugcggcccag

SEQ ID NO: 16 - RNA, 18 nt, Artificial Sequence
  si-MS8 antisense
cugggccgcaguggcugc

SEQ ID NO: 17 - RNA, 17 nt, Artificial Sequence
  si-MS9 sense
gcagcgcaugcggccca

SEQ ID NO: 18 - RNA, 17 nt, Artificial Sequence
  si-MS9 antisense
ugggccgcaguggcugc

SEQ ID NO: 19 - RNA, 21 nt, Artificial Sequence
  si-BB1 sense
aagaagaggagaaaaaaauga

SEQ ID NO: 20 - RNA, 21 nt, Artificial Sequence
  si-BB1 antisense
ucauuucuucucuuucuucuu

SEQ ID NO: 21 - RNA, 20 nt, Artificial Sequence
  si-BB2 sense
aagaagaggagaaaaaaaug

SEQ ID NO: 22 - RNA, 20 nt, Artificial Sequence
  si-BB2 antisense
cauuucuucucuuucuucuu

SEQ ID NO: 23 - RNA, 20 nt, Artificial Sequence
  si-BB3 sense
agaagaggagaaaaaaauga

SEQ ID NO: 24 - RNA, 20 nt, Artificial Sequence
  si-BB3 antisense
cauuucuucucuuucuucuu

SEQ ID NO: 25 - RNA, 19 nt, Artificial Sequence
  si-BB4 sense
gaagaggagaaaaaaauga

SEQ ID NO: 26 - RNA, 19 nt, Artificial Sequence
  si-BB4 antisense
ucauuucuucucuuucuuc

SEQ ID NO: 27 - RNA, 19 nt, Artificial Sequence
  si-BB5 sense
agaagaggagaaaaaaaug

SEQ ID NO: 28 - RNA, 19 nt, Artificial Sequence
  si-BB5 antisense
cauuucuucucuuucuucu

SEQ ID NO: 29 - RNA, 18 nt, Artificial Sequence
  si-BB6 sense
gaagaggagaaaaaaaug

SEQ ID NO: 30 - RNA, 18 nt, Artificial Sequence
  si-BB6 antisense
cauuucuucucuuucuuc

SEQ ID NO: 31 - RNA, 20 nt, Artificial Sequence
  si-AT1 sense
gcugcugcugcugccugggg

SEQ ID NO: 32 - RNA, 20 nt, Artificial Sequence
  si-AT1 antisense
ccccaugcagcugcagcagc

SEQ ID NO: 33 - RNA, 19 nt, Artificial Sequence
  si-AT2 sense
cugcugcugcugccugggg

SEQ ID NO: 34 - RNA, 19 nt, Artificial Sequence
  si-AT2 antisense
ccccaugcagcugcagcag

SEQ ID NO: 35 - RNA, 18 nt, Artificial Sequence
  si-AT3 sense
ugcugcugcugccugggg

SEQ ID NO: 36 - RNA, 18 nt, Artificial Sequence
  si-AT3 antisense
ccccaugcagcugcagca

SEQ ID NO: 37 - RNA, 17 nt, Artificial Sequence
  si-AT4 sense
gcugcugcugccugggg

SEQ ID NO: 38 - RNA, 17 nt, Artificial Sequence
  si-AT4 antisense
ccccaugcagcugcagc

SEQ ID NO: 39 - RNA, 19 nt, Artificial Sequence
  si-AT5 sense
ccacccccaccaccaccac

SEQ ID NO: 40 - RNA, 19 nt, Artificial Sequence
  si-AT5 antisense
gugguggcagcgguggugg

SEQ ID NO: 41 - RNA, 18 nt, Artificial Sequence
  si-AT6 sense
ccacccccaccaccacca

SEQ ID NO: 42 - RNA, 18 nt, Artificial Sequence
  si-AT6 antisense
ugguggcagcgguggugg

SEQ ID NO: 43 - RNA, 17 nt, Artificial Sequence
  si-AT7 sense
ccacccccaccaccacc

SEQ ID NO: 44 - RNA, 17 nt, Artificial Sequence
  si-AT7 antisense
gguggcagcgguggugg

SEQ ID NO: 45 - RNA, 23 nt, Artificial Sequence
  si-AT8 sense
uggaggcagagagugagagagaa

SEQ ID NO: 46 - RNA, 23 nt, Artificial Sequence
  si-AT8 antisense
uucucucagacgcucucccucca

SEQ ID NO: 47 - RNA, 22 nt, Artificial Sequence
  si-AT9 sense
ggaggcagagagugagagagaa

SEQ ID NO: 48 - RNA, 22 nt, Artificial Sequence
  si-AT9 antisense
uucucucagacgcucucccucc

SEQ ID NO: 49 - RNA, 22 nt, Artificial Sequence
  si-AT10 sense
uggaggcagagagugagagaga

SEQ ID NO: 50 - RNA, 22 nt, Artificial Sequence
  si-AT10 antisense
ucucucagacgcucucccucca

SEQ ID NO: 51 - RNA, 21 nt, Artificial Sequence
  si-AT11 sense
uggaggcagagagugagagag

SEQ ID NO: 52 - RNA, 21 nt, Artificial Sequence
  si-AT11 antisense
cucucagacgcucucccucca

SEQ ID NO: 53 - RNA, 20 nt, Artificial Sequence
  si-AT12 sense
ggaggcagagagugagagag

SEQ ID NO: 54 - RNA, 20 nt, Artificial Sequence
  si-AT12 antisense
cucucagacgcucucccucc

SEQ ID NO: 55 - RNA, 21 nt, Artificial Sequence
  si-AT13 sense
ggaggcagagagugagagaga

SEQ ID NO: 56 - RNA, 21 nt, Artificial Sequence
  si-AT13 antisense
ucucucagacgcucucccucc

SEQ ID NO: 57 - RNA, 19 nt, Artificial Sequence
  si-MM sense
gcagcuuggaggcagagcg

SEQ ID NO: 58 - RNA, 19 nt, Artificial Sequence
  si-MM antisense
cgcucucccuccaugcugc

SEQ ID NO: 59 - RNA, 19 nt, Artificial Sequence
  si-BM sense
gccaaggccacacagccaa

SEQ ID NO: 60 - RNA, 19 nt, Artificial Sequence
  si-BM antisense
uuggcuuuguguccuuggc

SEQ ID NO: 61 - RNA, 19 nt, Artificial Sequence
  si-ST sense
ccagccagacccagaagga

SEQ ID NO: 62 - RNA, 19 nt, Artificial Sequence
  si-ST antisense
uccuucuuggacaggcugg

SEQ ID NO: 63 - RNA, 19 nt, Artificial Sequence
  Dual-targeted siRNA (antisense c-MET)
accacacaucugacuuggu

SEQ ID NO: 64 - RNA, 19 nt, Artificial Sequence
  Dual-targeted siRNA (antisense PD-L1)
accaauucagcuguauggu

SEQ ID NO: 65 - DNA, 276 bp, Artificial Sequence
  U6 promoter
cctagagtcgacactagataacaacataggagctgtgattggctgttttcagccaatcagcactgactcatttgcatagcctttacaagcggtcacaaactcaagaaacgagcggttttaatagtcttttagaatattgtttatcgaaccgaataaggaactgtgctttgtgattcacatatcagtggaggggtgtggaaatggcaccttgatctcaccctcatcgaaagtggagttgatgtccttccctggctcgctacagacgcacttccgcaa

SEQ ID NO: 66 - DNA, 54 bp, Artificial Sequence
  MS-TTGGATCCAA loop shRNA
gactgtggcatccacctgcatttggatccaaatgcaggtaggcgcctcagtctt

SEQ ID NO: 67 - DNA, 54 bp, Artificial Sequence
  MS-TTCAAGAGAG loop shRNA
gactgtggcatccacctgcatttcaagagagatgcaggtaggcgcctcagtctt

SEQ ID NO: 68 - DNA, 54 bp, Artificial Sequence
  BB-TTGGATCCAA loop shRNA
aagaagaggagaaaaaaatgattggatccaatcatttcttctctttcttctttt

SEQ ID NO: 69 - DNA, 54 bp, Artificial Sequence
  BB-TTCAAGAGAG loop shRNA
aagaagaggagaaaaaaatgattcaagagagtcatttcttctctttcttctttt

SEQ ID NO: 70 - DNA, 52 bp, Artificial Sequence
  AT-TTGGATCCAA loop shRNA
gctgctgctgctgcctggggttggatccaaccccatgcagctgcagcagctt

SEQ ID NO: 71 - DNA, 52 bp, Artificial Sequence
  AT-TTCAAGAGAG loop shRNA
gctgctgctgctgcctggggttcaagagagccccatgcagctgcagcagctt

SEQ ID NO: 72 - DNA, 50 bp, Artificial Sequence
  c-MET/PD-L1-TTGGATCCAA loop shRNA coding sequence
accacacatctgacttggtttggatccaaaccaattcagctgtatggttt

SEQ ID NO: 73 - DNA, 50 bp, Artificial Sequence
  c-MET/PD-L1-TTCAAGAGAG loop shRNA coding sequence
accacacatctgacttggtttcaagagagaccaattcagctgtatggttt

SEQ ID NO: 74 - DNA, 455 bp, Artificial Sequence
  hTERT promoter
tggcccctccctcgggttaccccacagcctaggccgattcgacctctctccgctggggccctcgctggcgtccctgcaccctgggagcgcgagcggcgcgcgggcggggaagcgcggcccagacccccgggtccgcccggagcagctgcgctgtcggggccaggccgggctcccagtggattcgcgggcacagacgcccaggaccgcgctccccacgtggcggagggactggggacccgggcacccgtcctgccccttcaccttccagctccgcctcctccgcgcggaccccgccccgtcccgacccctcccgggtccccggcccagccccctccgggccctcccagcccctccccttcctttccgcggccccgccctctcctcgcggcgcgagtttcaggcagcgctgcgtcctgctgcgcacgtgggaagccctggccccggccacccccgcg

SEQ ID NO: 75 - DNA, 900 bp, Artificial Sequence
  E1A
acaccgggactgaaaatgagacatattatctgccacggaggtgttattaccgaagaaatggccgccagtcttttggaccagctgatcgaagaggtactggctgataatcttccacctcctagccattttgaaccacctacccttcacgaactgtatgatttagacgtgacggcccccgaagatcccaacgaggaggcggtttcgcagatttttcccgactctgtaatgttggcggtgcaggaagggattgacttactcacttttccgccggcgcccggttctccggagccgcctcacctttcccggcagcccgagcagccggagcagagagccttgggtccggtttctatgccaaaccttgtaccggaggtgatcgatcttacctgccacgaggctggctttccacccagtgacgacgaggatgaagagggtgaggagtttgtgttagattatgtggagcaccccgggcacggttgcaggtcttgtcattatcaccggaggaatacgggggacccagatattatgtgttcgctttgctatatgaggacctgtggcatgtttgtctacagtcctgtgtctgaacctgagcctgagcccgagccagaaccggagcctgcaagacctacccgccgtcctaaaatggcgcctgctatcctgagacgcccgacatcacctgtgtctagagaatgcaatagtagtacggatagctgtgactccggtccttctaacacacctcctgagatacacccggtggtcccgctgtgccccattaaaccagttgccgtgagagttggtgggcgtcgccaggctgtggaatgtatcgaggacttgcttaacgagcctgggcaacctttggacttgagctgtaaacgccccaggccataaggtgtaaacctgtga

SEQ ID NO: 76 - DNA, 572 bp, Artificial Sequence
  IRES
cccctctccctcccccccctaacgttactggccgaagccgcttggaataaggccggtgtgcgtttgtctatatgttattttccaccatattgccgtcttttggcaatgtgagggcccggaaacctggccctgtcttcttgacgagcattcctaggggtctttcccctctcgccaaaggaatgcaaggtctgttgaatgtcgtgaaggaagcagttcctctggaagcttcttgaagacaaacaacgtctgtagcgaccctttgcaggcagcggaaccccccacctggcgacaggtgcctctgcggccaaaagccacgtgtataagatacacctgcaaaggcggcacaaccccagtgccacgttgtgagttggatagttgtggaaagagtcaaatggctctcctcaagcgtattcaacaaggggctgaaggatgcccagaaggtaccccattgtatgggatctgatctggggcctcggtgcacatgctttacatgtgtttagtcgaggttaaaaaaacgtctaggccccccgaaccacggggacgtggttttcctttgaaaaacacgatgataa

SEQ ID NO: 77 - DNA, 1797 bp, Artificial Sequence
  E1B
catggaggcttgggagtgtttggaagatttttctgctgtgcgtaacttgctggaacagagctctaacagtacctcttggttttggaggtttctgtggggctcatcccaggcaaagttagtctgcagaattaaggaggattacaagtgggaatttgaagagcttttgaaatcctgtggtgagctgtttgattctttgaatctgggtcaccaggcgcttttccaagagaaggtcatcaagactttggatttttccacaccggggcgcgctgcggctgctgttgcttttttgagttttataaaggataaatggagcgaagaaacccatctgagcggggggtacctgctggattttctggccatgcatctgtggagagcggttgtgagacacaagaatcgcctgctactgttgtcttccgtccgcccggcgataataccgacggaggagcagcagcagcagcaggaggaagccaggcggcggcggcaggagcagagcccatggaacccgagagccggcctggaccctcgggaatgaatgttgtacaggtggctgaactgtatccagaactgagacgcattttgacaattacagaggatgggcaggggctaaagggggtaaagagggagcggggggcttgtgaggctacagaggaggctaggaatctagcttttagcttaatgaccagacaccgtcctgagtgtattacttttcaacagatcaaggataattgcgctaatgagcttgatctgctggcgcagaagtattccatagagcagctgaccacttactggctgcagccaggggatgattttgaggaggctattagggtatatgcaaaggtggcacttaggccagattgcaagtacaagatcagcaaacttgtaaatatcaggaattgttgctacatttctgggaacggggccgaggtggagatagatacggaggatagggtggcctttagatgtagcatgataaatatgtggccgggggtgcttggcatggacggggtggttattatgaatgtaaggtttactggccccaattttagcggtacggttttcctggccaataccaaccttatcctacacggtgtaagcttctatgggtttaacaatacctgtgtggaagcctggaccgatgtaagggttcggggctgtgccttttactgctgctggaagggggtggtgtgtcgccccaaaagcagggcttcaattaagaaatgcctctttgaaaggtgtaccttgggtatcctgtctgagggtaactccagggtgcgccacaatgtggcctccgactgtggttgcttcatgctagtgaaaagcgtggctgtgattaagcataacatggtatgtggcaactgcgaggacagggcctctcagatgctgacctgctcggacggcaactgtcacctgctgaagaccattcacgtagccagccactctcgcaaggcctggccagtgtttgagcataacatactgacccgctgttccttgcatttgggtaacaggaggggggtgttcctaccttaccaatgcaatttgagtcacactaagatattgcttgagcccgagagcatgtccaaggtgaacctgaacggggtgtttgacatgaccatgaagatctggaaggtgctgaggtacgatgagacccgcaccaggtgcagaccctgcgagtgtggcggtaaacatattaggaaccagcctgtgatgctggatgtgaccgaggagctgaggcccgatcacttggtgctggcctgcacccgcgctgagtttggctctagcgatgaagatacagattga

SEQ ID NO: 78 - DNA, 3762 bp, Artificial Sequence
  hTERT-E1A-IRES-E1B
tggcccctccctcgggttaccccacagcctaggccgattcgacctctctccgctggggccctcgctggcgtccctgcaccctgggagcgcgagcggcgcgcgggcggggaagcgcggcccagacccccgggtccgcccggagcagctgcgctgtcggggccaggccgggctcccagtggattcgcgggcacagacgcccaggaccgcgctccccacgtggcggagggactggggacccgggcacccgtcctgccccttcaccttccagctccgcctcctccgcgcggaccccgccccgtcccgacccctcccgggtccccggcccagccccctccgggccctcccagcccctccccttcctttccgcggccccgccctctcctcgcggcgcgagtttcaggcagcgctgcgtcctgctgcgcacgtgggaagccctggccccggccacccccgcgactagtacaccgggactgaaaatgagacatattatctgccacggaggtgttattaccgaagaaatggccgccagtcttttggaccagctgatcgaagaggtactggctgataatcttccacctcctagccattttgaaccacctacccttcacgaactgtatgatttagacgtgacggcccccgaagatcccaacgaggaggcggtttcgcagatttttcccgactctgtaatgttggcggtgcaggaagggattgacttactcacttttccgccggcgcccggttctccggagccgcctcacctttcccggcagcccgagcagccggagcagagagccttgggtccggtttctatgccaaaccttgtaccggaggtgatcgatcttacctgccacgaggctggctttccacccagtgacgacgaggatgaagagggtgaggagtttgtgttagattatgtggagcaccccgggcacggttgcaggtcttgtcattatcaccggaggaatacgggggacccagatattatgtgttcgctttgctatatgaggacctgtggcatgtttgtctacagtcctgtgtctgaacctgagcctgagcccgagccagaaccggagcctgcaagacctacccgccgtcctaaaatggcgcctgctatcctgagacgcccgacatcacctgtgtctagagaatgcaatagtagtacggatagctgtgactccggtccttctaacacacctcctgagatacacccggtggtcccgctgtgccccattaaaccagttgccgtgagagttggtgggcgtcgccaggctgtggaatgtatcgaggacttgcttaacgagcctgggcaacctttggacttgagctgtaaacgccccaggccataaggtgtaaacctgtgacccctctccctcccccccctaacgttactggccgaagccgcttggaataaggccggtgtgcgtttgtctatatgttattttccaccatattgccgtcttttggcaatgtgagggcccggaaacctggccctgtcttcttgacgagcattcctaggggtctttcccctctcgccaaaggaatgcaaggtctgttgaatgtcgtgaaggaagcagttcctctggaagcttcttgaagacaaacaacgtctgtagcgaccctttgcaggcagcggaaccccccacctggcgacaggtgcctctgcggccaaaagccacgtgtataagatacacctgcaaaggcggcacaaccccagtgccacgttgtgagttggatagttgtggaaagagtcaaatggctctcctcaagcgtattcaacaaggggctgaaggatgcccagaaggtaccccattgtatgggatctgatctggggcctcggtgcacatgctttacatgtgtttagtcgaggttaaaaaaacgtctaggccccccgaaccacggggacgtggttttcctttgaaaaacacgatgataagcttgccacaacccgggatcctctagagtcgacatggaggcttgggagtgtttggaagatttttctgctgtgcgtaacttgctggaacagagctctaacagtacctcttggttttggaggtttctgtggggctcatcccaggcaaagttagtctgcagaattaaggaggattacaagtgggaatttgaagagcttttgaaatcctgtggtgagctgtttgattctttgaatctgggtcaccaggcgcttttccaagagaaggtcatcaagactttggatttttccacaccggggcgcgctgcggctgctgttgcttttttgagttttataaaggataaatggagcgaagaaacccatctgagcggggggtacctgctggattttctggccatgcatctgtggagagcggttgtgagacacaagaatcgcctgctactgttgtcttccgtccgcccggcgataataccgacggaggagcagcagcagcagcaggaggaagccaggcggcggcggcaggagcagagcccatggaacccgagagccggcctggaccctcgggaatgaatgttgtacaggtggctgaactgtatccagaactgagacgcattttgacaattacagaggatgggcaggggctaaagggggtaaagagggagcggggggcttgtgaggctacagaggaggctaggaatctagcttttagcttaatgaccagacaccgtcctgagtgtattacttttcaacagatcaaggataattgcgctaatgagcttgatctgctggcgcagaagtattccatagagcagctgaccacttactggctgcagccaggggatgattttgaggaggctattagggtatatgcaaaggtggcacttaggccagattgcaagtacaagatcagcaaacttgtaaatatcaggaattgttgctacatttctgggaacggggccgaggtggagatagatacggaggatagggtggcctttagatgtagcatgataaatatgtggccgggggtgcttggcatggacggggtggttattatgaatgtaaggtttactggccccaattttagcggtacggttttcctggccaataccaaccttatcctacacggtgtaagcttctatgggtttaacaatacctgtgtggaagcctggaccgatgtaagggttcggggctgtgccttttactgctgctggaagggggtggtgtgtcgccccaaaagcagggcttcaattaagaaatgcctctttgaaaggtgtaccttgggtatcctgtctgagggtaactccagggtgcgccacaatgtggcctccgactgtggttgcttcatgctagtgaaaagcgtggctgtgattaagcataacatggtatgtggcaactgcgaggacagggcctctcagatgctgacctgctcggacggcaactgtcacctgctgaagaccattcacgtagccagccactctcgcaaggcctggccagtgtttgagcataacatactgacccgctgttccttgcatttgggtaacaggaggggggtgttcctaccttaccaatgcaatttgagtcacactaagatattgcttgagcccgagagcatgtccaaggtgaacctgaacggggtgtttgacatgaccatgaagatctggaaggtgctgaggtacgatgagacccgcaccaggtgcagaccctgcgagtgtggcggtaaacatattaggaaccagcctgtgatgctggatgtgaccgaggagctgaggcccgatcacttggtgctggcctgcacccgcgctgagtttggctctagcgatgaagatacagattga

SEQ ID NO: 79 - DNA, 319 bp, Artificial Sequence
  U6promoter-Bs-shRNA (CA101)
aaggtcgggcaggaagagggcctatttcccatgattccttcatatttgcatatacgatacaaggctgttagagagataattagaattaatttgactgtaaacacaaagatattagtacaaaatacgtgacgtagaaagtaataatttcttgggtagtttgcagttttaaaattatgttttaaaatggactatcatatgcttaccgtaacttgaaagtatttcgatttcttggctttatatatcttgtggaaaggacgaaacaccgaagaagaggagaaaaaaatgattcaagagagtcatttcttctctttcttctttt

SEQ ID NO: 80 - DNA, 317 bp, Artificial Sequence
  U6promoter-Bs-shRNA (CA102)
aaggtcgggcaggaagagggcctatttcccatgattccttcatatttgcatatacgatacaaggctgttagagagataattagaattaatttgactgtaaacacaaagatattagtacaaaatacgtgacgtagaaagtaataatttcttgggtagtttgcagttttaaaattatgttttaaaatggactatcatatgcttaccgtaacttgaaagtatttcgatttcttggctttatatatcttgtggaaaggacgaaacaccggactgtggcatccacctgcatttcaagagagatgcaggtaggcgcctcagtc

SEQ ID NO: 81 - DNA, 315 bp, Artificial Sequence
  U6promoter-Bs-shRNA (CA103)
aaggtcgggcaggaagagggcctatttcccatgattccttcatatttgcatatacgatacaaggctgttagagagataattagaattaatttgactgtaaacacaaagatattagtacaaaatacgtgacgtagaaagtaataatttcttgggtagtttgcagttttaaaattatgttttaaaatggactatcatatgcttaccgtaacttgaaagtatttcgatttcttggctttatatatcttgtggaaaggacgaaacaccggctgctgctgctgcctggggttcaagagagccccatgcagctgcagcagc

SEQ ID NO: 82 - DNA, 483 bp, Artificial Sequence
  E3 DEL
atgattaggtacataatcctaggtttactcacccttgcgtcagcccacggtaccacccaaaaggtggattttaaggagccagcctgtaatgttacattcgcagctgaagctaatgagtgcaccactcttataaaatgcaccacagaacatgaaaagctgcttattcgccacaaaaacaaaattggcaagtatgctgtttatgctatttggcagccaggtgacactacagagtataatgttacagttttccagggtaaaagtcataaaacttttatgtatacttttccattttatgaaatgtgcgacattaccatgtacatgagcaaacagtataagttgtggcccccacaaaattgtgtggaaaacactggcactttctgctgcactgctatgctaattacagtgctcgctttggtctgtaccctactctatattaaatacaaaagcagacgcagctttattgaggaaaagaaaatgccttaa